European Patent Application EP 4 545 551 A1, published April 30, 2025. Title: Peptide inhibitors and uses thereof. Applicant: 成都倍特新启生物医药有限责任公司. The sequence listing filed with the application follows.

SEQUENCE LISTING (51 sequences)

SEQ ID NO: 1 - protein, 5 aa, synthetic construct
  REGION 1..5: note = synthetic
  MOD_RES 1: note = ACETYLATION
  MOD_RES 5: note = AMIDATION
QDPED

SEQ ID NO: 2 - protein, 5 aa, synthetic construct
  REGION 1..5: note = synthetic
  MOD_RES 1: note = ACETYLATION
  MOD_RES 5: note = AMIDATION
QDAED

SEQ ID NO: 3 - protein, 6 aa, synthetic construct
  REGION 1..6: note = synthetic
  MOD_RES 1: note = ACETYLATION
  MOD_RES 6: note = AMIDATION
TQDPED

SEQ ID NO: 4 - protein, 6 aa, synthetic construct
  REGION 1..6: note = synthetic
  MOD_RES 1: note = ACETYLATION
  MOD_RES 6: note = AMIDATION
TQDAED

SEQ ID NO: 5 - protein, 6 aa, synthetic construct
  REGION 1..6: note = synthetic
  MOD_RES 1: note = ACETYLATION
  MOD_RES 6: note = AMIDATION
QDAEDN

SEQ ID NO: 6 - protein, 7 aa, synthetic construct
  REGION 1..7: note = synthetic
  MOD_RES 1: note = ACETYLATION
  MOD_RES 7: note = AMIDATION
TQDAEDN

SEQ ID NO: 7 - protein, 7 aa, synthetic construct
  REGION 1..7: note = synthetic
  MOD_RES 1: note = ACETYLATION
  MOD_RES 7: note = AMIDATION
SQDAEDN

SEQ ID NO: 8 - protein, 7 aa, synthetic construct
  REGION 1..7: note = synthetic
  MOD_RES 1: note = ACETYLATION
  MOD_RES 7: note = AMIDATION
TNDAEDN

SEQ ID NO: 9 - protein, 7 aa, synthetic construct
  REGION 1..7: note = synthetic
  MOD_RES 1: note = ACETYLATION
  MOD_RES 7: note = AMIDATION
TEDAEDN

SEQ ID NO: 10 - protein, 7 aa, synthetic construct
  REGION 1..7: note = synthetic
  MOD_RES 1: note = ACETYLATION
  MOD_RES 7: note = AMIDATION
TSDAEDN

SEQ ID NO: 11 - protein, 7 aa, synthetic construct
  REGION 1..7: note = synthetic
  MOD_RES 1: note = ACETYLATION
  MOD_RES 7: note = AMIDATION
TQDSEDN

SEQ ID NO: 12 - protein, 7 aa, synthetic construct
  REGION 1..7: note = synthetic
  MOD_RES 1: note = ACETYLATION
  MOD_RES 7: note = AMIDATION
TQDAEDL

SEQ ID NO: 13 - protein, 7 aa, synthetic construct
  REGION 1..7: note = synthetic
  MOD_RES 1: note = ACETYLATION
  MOD_RES 7: note = AMIDATION
TQDAEDP

SEQ ID NO: 14 - protein, 7 aa, synthetic construct
  REGION 1..7: note = synthetic
  MOD_RES 1: note = ACETYLATION
  MOD_RES 7: note = AMIDATION
TQDPEDN

SEQ ID NO: 15 - protein, 8 aa, synthetic construct
  REGION 1..8: note = synthetic
  MOD_RES 1: note = ACETYLATION
  MOD_RES 8: note = AMIDATION
TQDAEDNT

SEQ ID NO: 16 - protein, 8 aa, synthetic construct
  REGION 1..8: note = synthetic
  MOD_RES 1: note = ACETYLATION
  MOD_RES 8: note = AMIDATION
QDAEDNTA

SEQ ID NO: 17 - protein, 9 aa, synthetic construct
  REGION 1..9: note = synthetic
  MOD_RES 1: note = ACETYLATION
  MOD_RES 9: note = AMIDATION
TQDAEDNTV

SEQ ID NO: 18 - protein, 9 aa, synthetic construct
  REGION 1..9: note = synthetic
  MOD_RES 1: note = ACETYLATION
  MOD_RES 9: note = AMIDATION
SQDAEDNTV

SEQ ID NO: 19 - protein, 9 aa, synthetic construct
  REGION 1..9: note = synthetic
  MOD_RES 1: note = ACETYLATION
  MOD_RES 9: note = AMIDATION
TNDAEDNTV

SEQ ID NO: 20 - protein, 9 aa, synthetic construct
  REGION 1..9: note = synthetic
  MOD_RES 1: note = ACETYLATION
  MOD_RES 9: note = AMIDATION
TQDPEDNTV

SEQ ID NO: 21 - protein, 9 aa, synthetic construct
  REGION 1..9: note = synthetic
  MOD_RES 1: note = ACETYLATION
  MOD_RES 9: note = AMIDATION
TQDSEDNTV

SEQ ID NO: 22 - protein, 9 aa, synthetic construct
  REGION 1..9: note = synthetic
  MOD_RES 1: note = ACETYLATION
  MOD_RES 9: note = AMIDATION
TQDAEDPTA

SEQ ID NO: 23 - protein, 9 aa, synthetic construct
  REGION 1..9: note = synthetic
  MOD_RES 1: note = ACETYLATION
  MOD_RES 9: note = AMIDATION
QDAEDNTAS

SEQ ID NO: 24 - protein, 10 aa, synthetic construct
  REGION 1..10: note = synthetic
  MOD_RES 1: note = ACETYLATION
  MOD_RES 10: note = AMIDATION
TQDAEDNTAS

SEQ ID NO: 25 - protein, 10 aa, synthetic construct
  REGION 1..10: note = synthetic
  MOD_RES 1: note = ACETYLATION
  MOD_RES 10: note = AMIDATION
TQDAEDPTAS

SEQ ID NO: 26 - protein, 10 aa, synthetic construct
  REGION 1..10: note = synthetic
  MOD_RES 1: note = ACETYLATION
  MOD_RES 10: note = AMIDATION
TQDPEDNTAS

SEQ ID NO: 27 - protein, 11 aa, synthetic construct
  REGION 1..11: note = synthetic
  MOD_RES 1: note = ACETYLATION
  MOD_RES 11: note = AMIDATION
TQDAEDNTVSF

SEQ ID NO: 28 - protein, 11 aa, synthetic construct
  REGION 1..11: note = synthetic
  MOD_RES 1: note = ACETYLATION
  MOD_RES 11: note = AMIDATION
SQDAEDNTVSF

SEQ ID NO: 29 - protein, 11 aa, synthetic construct
  REGION 1..11: note = synthetic
  MOD_RES 1: note = ACETYLATION
  MOD_RES 11: note = AMIDATION
TEDAEDNTVSF

SEQ ID NO: 30 - protein, 11 aa, synthetic construct
  REGION 1..11: note = synthetic
  MOD_RES 1: note = ACETYLATION
  MOD_RES 11: note = AMIDATION
TQDPEDNTVSF

SEQ ID NO: 31 - protein, 11 aa, synthetic construct
  REGION 1..11: note = synthetic
  MOD_RES 1: note = ACETYLATION
  MOD_RES 11: note = AMIDATION
TQDAEDNTASF

SEQ ID NO: 32 - protein, 11 aa, synthetic construct
  REGION 1..11: note = synthetic
  MOD_RES 1: note = ACETYLATION
  MOD_RES 11: note = AMIDATION
TQDAEDNTASY

SEQ ID NO: 33 - protein, 11 aa, synthetic construct
  REGION 1..11: note = synthetic
  MOD_RES 1: note = ACETYLATION
  MOD_RES 11: note = AMIDATION
TQDAEDNTASH

SEQ ID NO: 34 - protein, 11 aa, synthetic construct
  REGION 1..11: note = synthetic
  MOD_RES 1: note = ACETYLATION
  MOD_RES 11: note = AMIDATION
TQDAEDNTASW

SEQ ID NO: 35 - protein, 12 aa, synthetic construct
  REGION 1..12: note = synthetic
  MOD_RES 1: note = ACETYLATION
  MOD_RES 12: note = AMIDATION
TQDAEDNTASHL

SEQ ID NO: 36 - protein, 13 aa, synthetic construct
  REGION 1..13: note = synthetic
  MOD_RES 1: note = ACETYLATION
  MOD_RES 13: note = AMIDATION
TQDAEDNTVSFLQ

SEQ ID NO: 37 - protein, 13 aa, synthetic construct
  REGION 1..13: note = synthetic
  MOD_RES 1: note = ACETYLATION
  MOD_RES 13: note = AMIDATION
SQDAEDNTVSFLQ

SEQ ID NO: 38 - protein, 13 aa, synthetic construct
  REGION 1..13: note = synthetic
  MOD_RES 1: note = ACETYLATION
  MOD_RES 13: note = AMIDATION
TSDAEDNTVSFLQ

SEQ ID NO: 39 - protein, 13 aa, synthetic construct
  REGION 1..13: note = synthetic
  MOD_RES 1: note = ACETYLATION
  MOD_RES 13: note = AMIDATION
TQDPEDNTVSFLQ

SEQ ID NO: 40 - protein, 7 aa, synthetic construct
  REGION 1..7: note = synthetic
  REGION 1..7: note = MISC_FEATURE - head-to-tail backbone cyclization
TQDAEDN

SEQ ID NO: 41 - protein, 7 aa, synthetic construct
  REGION 1..7: note = synthetic
  REGION 1..7: note = MISC_FEATURE - head-to-tail backbone cyclization
TQDPEDN

SEQ ID NO: 42 - protein, 8 aa, synthetic construct
  REGION 1..8: note = synthetic
  REGION 3..8: note = MISC_FEATURE - Lactam bridge
TQDAEDNK

SEQ ID NO: 43 - protein, 8 aa, synthetic construct
  REGION 1..8: note = synthetic
  MOD_RES 1: note = ACETYLATION
  REGION 2..8: note = MISC_FEATURE - disulfide-bridge
TCDAEDNC

SEQ ID NO: 44 - protein, 8 aa, synthetic construct
  REGION 1..8: note = synthetic
  MOD_RES 1: note = ACETYLATION
  REGION 2..8: note = MISC_FEATURE - disulfide bridge
  MOD_RES 8: note = AMIDATION
TCDAEDNC

SEQ ID NO: 45 - protein, 7 aa, synthetic construct
  REGION 1..7: note = synthetic
  REGION 1..7: note = MISC_FEATURE - head to tail backbone cyclization
QDAEDNT

SEQ ID NO: 46 - protein, 10 aa, synthetic construct
  REGION 1..10: note = synthetic
  REGION 1..10: note = MISC_FEATURE - head to tail backbon cyclization
TQDPEDNTAS

SEQ ID NO: 47 - protein, 7 aa, synthetic construct
  REGION 1..7: note = synthetic
  MOD_RES 1: note = ACETYLATION
  MOD_RES 7: note = AMIDATION
TQDPAED

SEQ ID NO: 48 - protein, 8 aa, synthetic construct
  REGION 1..8: note = synthetic
  MOD_RES 1: note = ACETYLATION
  MOD_RES 8: note = AMIDATION
TQDPAEDN

SEQ ID NO: 49 - protein, 10 aa, synthetic construct
  REGION 1..10: note = synthetic
  MOD_RES 1: note = ACETYLATION
  MOD_RES 10: note = AMIDATION
TQDAEDNTQD

SEQ ID NO: 50 - protein, 18 aa, synthetic construct
  REGION 1..18: note = synthetic
YRVRFLAKENVTQDAEDN

SEQ ID NO: 51 - protein, 13 aa, synthetic construct
  REGION 1..13: note = synthetic
TQDAEDNTVSFLQ